European Patent Specification EP 3 624 838 B1, published January 25, 2023. Title: METHODS OF USE OF SOLUBLE CD24 FOR NEUROPROTECTION AND REMYELINATION. Applicant: OncoImmune, Inc. Children's National Medical Center Liu, Yang Zheng, Pan Li, Ning Devenport, Martin. The sequence listing filed with the application follows.

SEQUENCE LISTING (12 sequences)

SEQ ID NO: 1 - protein, 31 aa, Homo sapiens
  VARIANT (31)...(31): Valine or Alanine
SETTTGTSSNSSQSTSNSGLAPNPTNATTKX

SEQ ID NO: 2 - protein, 30 aa, Homo sapiens
SETTTGTSSNSSQSTSNSGLAPNPTNATTK

SEQ ID NO: 3 - protein, 27 aa, Mus musculus
NQTSVAPFPGNQNISASPNPTNATTRG

SEQ ID NO: 4 - protein, 26 aa, Homo sapiens
MGRAMVARLGLGLLLLALLLPTQIYS

SEQ ID NO: 5 - protein, 287 aa, Artificial
  Fusion protein
MGRAMVARLGLGLLLLALLLPTQIYSSETTTGTSSNSSQSTSNSGLAPNPTNATTKPKSCDKTHTCPPCPAPELLGGPSVFLFPPKPKDTLMISRTPEVTCVVVDVSHEDPEVKFNWYVDGVEVHNAKTKPREEQYNSTYRVVSVLTVLHQDWLNGKEYKCKVSNKALPAPIEKTISKAKGQPREPQVYTLPPSRDELTKNQVSLTCLVKGFYPSDIAVEWESNGQPENNYKTTPPVLDSDGSFFLYSKLTVDKSRWQQGNVFSCSVMHEALHNHYTQKSLSLSPGK

SEQ ID NO: 6 - protein, 261 aa, Artificial
  Fusion protein
SETTTGTSSNSSQSTSNSGLAPNPTNATTKPKSCDKTHTCPPCPAPELLGGPSVFLFPPKPKDTLMISRTPEVTCVVVDVSHEDPEVKFNWYVDGVEVHNAKTKPREEQYNSTYRVVSVLTVLHQDWLNGKEYKCKVSNKALPAPIEKTISKAKGQPREPQVYTLPPSRDELTKNQVSLTCLVKGFYPSDIAVEWESNGQPENNYKTTPPVLDSDGSFFLYSKLTVDKSRWQQGNVFSCSVMHEALHNHYTQKSLSLSPGK

SEQ ID NO: 7 - protein, 231 aa, Homo sapiens
PKSCDKTHTCPPCPAPELLGGPSVFLFPPKPKDTLMISRTPEVTCVVVDVSHEDPEVKFNWYVDGVEVHNAKTKPREEQYNSTYRVVSVLTVLHQDWLNGKEYKCKVSNKALPAPIEKTISKAKGQPREPQVYTLPPSRDELTKNQVSLTCLVKGFYPSDIAVEWESNGQPENNYKTTPPVLDSDGSFFLYSKLTVDKSRWQQGNVFSCSVMHEALHNHYTQKSLSLSPGK

SEQ ID NO: 8 - protein, 288 aa, Artificial
  Fusion protein
MGRAMVARLGLGLLLLALLLPTQIYSSETTTGTSSNSSQSTSNSGLAPNPTNATTKVPKSCDKTHTCPPCPAPELLGGPSVFLFPPKPKDTLMISRTPEVTCVVVDVSHEDPEVKFNWYVDGVEVHNAKTKPREEQYNSTYRVVSVLTVLHQDWLNGKEYKCKVSNKALPAPIEKTISKAKGQPREPQVYTLPPSRDELTKNQVSLTCLVKGFYPSDIAVEWESNGQPENNYKTTPPVLDSDGSFFLYSKLTVDKSRWQQGNVFSCSVMHEALHNHYTQKSLSLSPGK

SEQ ID NO: 9 - protein, 288 aa, Artificial
  Fusion protein
MGRAMVARLGLGLLLLALLLPTQIYSSETTTGTSSNSSQSTSNSGLAPNPTNATTKAPKSCDKTHTCPPCPAPELLGGPSVFLFPPKPKDTLMISRTPEVTCVVVDVSHEDPEVKFNWYVDGVEVHNAKTKPREEQYNSTYRVVSVLTVLHQDWLNGKEYKCKVSNKALPAPIEKTISKAKGQPREPQVYTLPPSRDELTKNQVSLTCLVKGFYPSDIAVEWESNGQPENNYKTTPPVLDSDGSFFLYSKLTVDKSRWQQGNVFSCSVMHEALHNHYTQKSLSLSPGK

SEQ ID NO: 10 - protein, 29 aa, Macaca fascicularis
TVTTSAPLSSNSPQNTSTTPNPANTTTKA

SEQ ID NO: 11 - protein, 262 aa, Artificial
  Fusion protein
SETTTGTSSNSSQSTSNSGLAPNPTNATTKVPKSCDKTHTCPPCPAPELLGGPSVFLFPPKPKDTLMISRTPEVTCVVVDVSHEDPEVKFNWYVDGVEVHNAKTKPREEQYNSTYRVVSVLTVLHQDWLNGKEYKCKVSNKALPAPIEKTISKAKGQPREPQVYTLPPSRDELTKNQVSLTCLVKGFYPSDIAVEWESNGQPENNYKTTPPVLDSDGSFFLYSKLTVDKSRWQQGNVFSCSVMHEALHNHYTQKSLSLSPGK

SEQ ID NO: 12 - protein, 262 aa, Artificial
  Fusion protein
SETTTGTSSNSSQSTSNSGLAPNPTNATTKAPKSCDKTHTCPPCPAPELLGGPSVFLFPPKPKDTLMISRTPEVTCVVVDVSHEDPEVKFNWYVDGVEVHNAKTKPREEQYNSTYRVVSVLTVLHQDWLNGKEYKCKVSNKALPAPIEKTISKAKGQPREPQVYTLPPSRDELTKNQVSLTCLVKGFYPSDIAVEWESNGQPENNYKTTPPVLDSDGSFFLYSKLTVDKSRWQQGNVFSCSVMHEALHNHYTQKSLSLSPGK